European Patent Application EP 4 349 974 A1, published April 10, 2024. Title: Method for producing reassortant rotavirus. Applicant: SK bioscience Co., Ltd. The sequence listing filed with the application follows.

SEQUENCE LISTING (18 sequences)

SEQ ID NO: 1 - DNA, 1062 bp, Rotavirus strain WC3
  gene (1)..(1062): V7 gene segment (AY050272)
ggctttaaaagagagaatttccgtctggctagcggttagctccttttaatgtatggtattgaatataccacaattctaatcttcttgacatcgattacattattaaattatatcttaaaatcaataacgagaataatggactatataatttatagatttttgcttatggtagtgatcttggccaccataataaatgcgcaaaactatggagtaaatttgccaattacaggttcaatggatactgcgtatgcaaactctacacaaagtgagccatttttgacatcaaccctttgtttgtattatcctgttgaggcatcaaacgaaatagctgatactgaatggaaagataccttatcacaactgttcttaacaaaaggatggccaacaggatcagtgtactttaaagaatatgctgatatagcggccttttcagtggaaccacagttatactgtgattataatttagttttaatgaaatatgactctacacaaaaactagatatgtctgaattggccgatcttatattgaatgaatggctgtgcaatccaatggacataacgctatattattatcagcagactgatgaggcaaataaatggatatcgatgggctcttcttgcaacgttaaagtgtgtccattaaatacacaaacacttggtattggatgtctaataactaatccagacacgtttgaaacagttgcgacaacggagaaattagtgattacagatgttgtagatggtgtcaaccacaaattaaacgtcacaacggcaacgtgcaccatacgcaactgtaaaaagttaggaccaagggagaacgtagcagtcatacaggtaggcggcgcgaacattttagacatcacagctgatccaacaactacaccacagacagagagaatgatgcgaataaattggaaaaaatggtggcaatgtttttacacggtagtggattacgtcaatcaaataattcagacagtatccaaaagatctagatcgcttaattcgtcggcgttctactatagagtgtaggtgcatcttagattagaattgtatgatgtgacc

SEQ ID NO: 2 - DNA, 1062 bp, Rotavirus strain Brb9
  gene (1)..(1062): VP7 gene segment (GU565090)
ggctttaaaagagagaatttccgtttggctagcggatagctccttttaatgtatggtattgaatataccacagttctattttatttgatatcgttcgttcttgtgagttatattctgaaaactatgataaagataatggactatttaatttatagaataacatttgtaattgtagtattatcagtattatcgaatgcacaaaattatggaataaatttgccaattactggatctatggatacagcatatgctaactcaacacaagacaataattttttatcttcaactttatgtctatattatccatcagaagctccaactcaaattagtgacactgaatggaaagatacactatctcaactgtttttaaccaaaggatggccgacaggttcagtttattttaatgaatattcaaacgttttagaattttccatcgacccaaagctatactgtgattataatgttgtgttaattagattcgcttctggtgaggagttggacgtatctgaattagctgatctaatactcaatgagtggttatgtaatccaatggatataacattatattattatcaacaaactggagaggcaaataagtggatatcaatgggatcatcatgtaccgttaaagtgtgtccattaaatactcagacattaggaattggatgtcaaacgacagatactgctacttttgaaacagttgctgacagcgaaaaattggcattaattgatgttgttgacaacgtaaatcataaattagatgttacatctactacgtgtacaatacggaattgtaataaactaggacctagagaaaatgtggctataatacaggttggcggttctaatatattagatataacagctgatcccacaacttctccacaaacagaacgaatgatgcgcgtaaactggaaaaaatggtggcaagtattctatactgtagttgattacattaatcaaatagtaaaagtaatgtccaaaagatcaagatcgttagattcgtcatctttctattatagagtatagatatatcctaaaatagaactgtttgatgtgacc

SEQ ID NO: 3 - DNA, 21 bp, Artificial Sequence
  miRNA target site 1
caattctaatcttcttgacat

SEQ ID NO: 4 - DNA, 21 bp, Artificial Sequence
  miRNA target site 2
ttgtttgtattatcctgttga

SEQ ID NO: 5 - DNA, 21 bp, Artificial Sequence
  miRNA target site 3
tggtgtcaaccacaaattaaa

SEQ ID NO: 6 - DNA, 64 bp, Artificial Sequence
  pre-miRNA top strand against target site 1
tgctgatgtcaagaagattagaattggttttggccactgactgaccaattctacttcttgacat

SEQ ID NO: 7 - DNA, 64 bp, Artificial Sequence
  pre-miRNA bottom strand against target site 1
cctgatgtcaagaagtagaattggtcagtcagtggccaaaaccaattctaatcttcttgacatc

SEQ ID NO: 8 - DNA, 64 bp, Artificial Sequence
  pre-miRNA top strand against target site 2
tgctgtcaacaggataatacaaacaagttttggccactgactgacttgtttgttatcctgttga

SEQ ID NO: 9 - DNA, 64 bp, Artificial Sequence
  pre-miRNA bottom strand against target site 2
cctgtcaacaggataacaaacaagtcagtcagtggccaaaacttgtttgtattatcctgttgac

SEQ ID NO: 10 - DNA, 64 bp, Artificial Sequence
  pre-miRNA top strand against target site 3
tgctgtttaatttgtggttgacaccagttttggccactgactgactggtgtcacacaaattaaa

SEQ ID NO: 11 - DNA, 64 bp, Artificial Sequence
  pre-miRNA bottom strand against target site 3
cctgtttaatttgtgtgacaccagtcagtcagtggccaaaactggtgtcaaccacaaattaaac

SEQ ID NO: 12 - DNA, 1228 bp, Artificial Sequence
  DNA template for BrB9 VP7 mRNA in vitro transcription
gaattctaatacgactcactactataggctttaaaagagagaatttccgtttggctagcggatagctccttttaatgtatggtattgaatataccacagttctattttatttgatatcgttcgttcttgtgagttatattctgaaaactatgataaagataatggactatttaatttatagaataacatttgtaattgtagtattatcagtattatcgaatgcacaaaattatggaataaatttgccaattactggatctatggatacagcatatgctaactcaacacaagacaataattttttatcttcaactttatgtctatattatccatcagaagctccaactcaaattagtgacactgaatggaaagatacactatctcaactgtttttaaccaaaggatggccgacaggttcagtttattttaatgaatattcaaacgttttagaattttccatcgacccaaagctatactgtgattataatgttgtgttaattagattcgcttctggtgaggagttggacgtatctgaattagctgatctaatactcaatgagtggttatgtaatccaatggatataacattatattattatcaacaaactggagaggcaaataagtggatatcaatgggatcatcatgtaccgttaaagtgtgtccattaaatactcagacattaggaattggatgtcaaacgacagatactgctacttttgaaacagttgctgacagcgaaaaattggcattaattgatgttgttgacaacgtaaatcataaattagatgttacatctactacgtgtacaatacggaattgtaataaactaggacctagagaaaatgtggctataatacaggttggcggttctaatatattagatataacagctgatcccacaacttctccacaaacagaacgaatgatgcgcgtaaactggaaaaaatggtggcaagtattctatactgtagttgattacattaatcaaatagtaaaagtaatgtccaaaagatcaagatcgttagattcgtcatctttctattatagagtatagatatatcctaaaatagaactgtttgatgtgaccgggtcggcatggtcccagcctcctcgctggcgccggctgggcaacattccgaggggaccgtcccctcggtaatggcgaatgggacgcatagcataaccccttggggcctctaaacgggtcttgaggggttttttggatcc

SEQ ID NO: 13 - DNA, 25 bp, Artificial Sequence
  WC3V7_F primer
tcttgacatcgattacattattaaa

SEQ ID NO: 14 - DNA, 29 bp, Artificial Sequence
  WC3V7_R primer
catatctagtttttgtgtagagtcatatt

SEQ ID NO: 15 - DNA, 24 bp, Artificial Sequence
  Brb9V7_F primer
ttcgttcttgtgagttatattctg

SEQ ID NO: 16 - DNA, 20 bp, Artificial Sequence
  Brb9V7_R primer
gtccaactcctcaccagaag

SEQ ID NO: 17 - DNA, 22 bp, Artificial Sequence
  WC3V4_F primer
gtcgttcgatctaccagtagga

SEQ ID NO: 18 - DNA, 25 bp, Artificial Sequence
  WC3V4_R primer
gtcactatatggccttacctcaact